European Patent Application EP 4 389 895 A1, published June 26, 2024. Title: Mammalian Artificial Chromosome Vector having Immunoglobulin Heavy Chain Locus with Modified D Segment, and Cells and Non-human animals comprising Same. Applicant: National University Corporation Tottori University. The sequence listing filed with the application follows.

SEQUENCE LISTING (175 sequences)

SEQ ID NO: 1 - DNA, 8974 bp, synthetic construct
  misc_feature 1..8974: note = nucleotide sequence of human minimized D region
  misc_feature 647..663: note = D1-1
  misc_feature 920..950: note = D2-2
  misc_feature 1207..1237: note = D3-3
  misc_feature 1494..1509: note = D4-4
  misc_feature 1766..1785: note = D5-5
  misc_feature 2042..2059: note = D6-6
  misc_feature 2316..2332: note = D1-7
  misc_feature 2589..2619: note = D2-8
  misc_feature 2875..2905: note = D3-9
  misc_feature 3059..3089: note = D3-10
  misc_feature 3406..3421: note = D4-11
  misc_feature 3678..3700: note = D5-12
  misc_feature 3957..3977: note = D6-13
  misc_feature 4237..4253: note = D1-14
  misc_feature 4510..4540: note = D2-15
  misc_feature 4797..4833: note = D3-16
  misc_feature 5090..5105: note = D4-17
  misc_feature 5362..5381: note = D5-18
  misc_feature 5638..5658: note = D6-19
  misc_feature 5915..5931: note = D1-20
  misc_feature 6188..6215: note = D2-21
  misc_feature 6472..6502: note = D3-22
  misc_feature 6819..6837: note = D4-23
  misc_feature 7094..7113: note = D5-24
  misc_feature 7370..7387: note = D6-25
  misc_feature 7644..7663: note = D1-26
  source 1..8974: mol_type = other DNA
gtcgcctctacgggaaatccgggactcagcagtaaccctcaggaagcagggcccaggcgccgtttaataggaggcttcctcacaatgaaacttttagaaagccttgactacaatgatgaccttggtgtggctgtgaacactgtcagctcccacagctgctgcagcaaaaaatgtccatagacagggtgggggcccggggtcgtctgctgtcctgctcagcccacagcacgcatggaggatctgaggtgccacacctgacgcccaggccagaacatgcctccctccagggtgacctgccatgtcctgcattgctggagggacaggggcagcctatgaggatctggggccaggagatgaatcctattaacccagaggaaaactaacaggacccaagcaccctccccgttgaagctgacctgcccagaggggcctgggcccaccccacacaccggggcggaatgtgtacaggccccggtctctgtgggtgttccgctaactggggctcccagtgctcaccccacaactaaagcgagccccagcctccagagcccccgaaggagatgccgcccacaagcccagcccccatccaggaggccccagagctcagggcgccggggcagattctgaacagccccgagtcacggtgggtacaactggaacgaccaccgtgagaaaaactgtgtccaaaactctctcctggcccctgctggaggccgcgccagagaggggagcagccgccccgaacctaggtcctgctcagctcacacgacccccagcagccagagcacagtccctgagtttcagacaaaaaccccctggaaatcatagtatcagcaggagaactagccagagacagcaagaggggactcagtgactcccgcggggacaggaggattttgtgggggctcgtgtcactgtgaggatattgtagtagtaccagctgctatgcccacagtgacacagccccattcccaaagccctgctgtaaacgcttccacttctggagctgaggggctggggggagcgtctgggaagtagggcctaggggtggccatcaatgcccaaaacgcaccagactcagtagacctgagagcgctgggcccacagcctcccctcggtgccctgctacctcctcaggtcagccctggacatcccgggtttccccaggcctggcggtaggtttggggtgaggtctgtgtcactgtggtattacgatttttggagtggttattatacccacagtgtcacagagtccatcaaaaacccatccctgggaaccttctgccacagccctccctgtggggcaccgctgcgtgccatgttaggattttgactgaggacacagcaccatgggtatggtggctagaaaggtctgagatccccaggacgcagcaccactgtcaatgggggccccagacgcctggaccagggcctgcgtgggaaaggcctctgggcacactcaggggctttttgtgaagggtcctcctactgtgtgactacagtaactaccacagtgatgaacccagcagcaaaaactgaccggactcccaaggtttatgcacacttctccgctcagagctctccaggatcagaagagccgggcccaagggtttctgcccagaccctcggcctctaggccccatgtccccagtcctgggggcccctggcacagctgtctggaccctctctattccctgggaagctcctcctgacagccccgcctccagttccaggtgtggttattgtcagggggtgtcagactgtggtggatacagctatggttaccacagtggtgctgcccatagcagcaaccaggccaagtagacaggcccctgctgtgcagccccaggcctccagctcacctgcttctcctggggctctcaaggctgctgttttctgcactctcccctctgggcaggccccccagaaccagggatgaggacgccccgtcaaggccagaaaagaccaagttgtgctgagcccagcaagggaaggtccccaaacaaaccaggaagtttctgaaggtgtctgtgtcacagtggagtatagcagctcgtcccacagtgacactcgccaggccagaaaccccatcccaagtcagcggaatgcagagagagcagggaggacatgtttaggatctgaggccgcacctgacacccaggccagcagacgtctcctgtccatggcccacacctaaaacgagccacagcctcagagcccctgaaggagaccccgcccacaagcccagcccccacccaggaggccccagagcacagggcgccccgtcggattctgaacagccccgagtcacagtgggtataactggaactaccactgtgagaaaagcttcgtccaaaacggtctcctggccacagtcggaggccccgccagagaggggagcagccaccccaaacccatgttctgccggctcccatgaccccgtgcacctggagccccacacccagagtttcagacaaaaaccccctggaatgcacagtctcagcaggagagccagccagagccagcaagatggggctcagtgacacccgcagggacaggaggattttgtgggggctcgtgtcactgtgaggatattgtactaatggtgtatgctatacccacagtgacacagccccattcccaaagccctactgcaaacgcattccacttctggggctgaggggctgggggagcgtctgggaaatagggctcaggggtgtccatcaatgcccaaaacgcaccagaccagcagacctgagagcgctgggcccacagcctcccctcagagccctgctgcctcctccggtcagccctggacatcccaggtttccccaggcctgccggtaggtttagaatgaggtctgtgtcactgtggtattacgatattttgactggttattataaccacagtgtcacagagtccatcaaaaacccatgcctggaagcttcccgccacagccctccccatggggccctgctgcctcctcaggtcagccccggacatcccgggtttccccaggctgggcggtaggtttggggtgaggtctgtgtcactgtggtattactatggttcggggagttattataaccacagtgtcacagagtccatcaaaaacccatccctgggagcctcccgccacagccctccctgcaggggaccggtacgtgccatgttaggattttgatcgaggagacagcaccatgggtatggtggctaatgcatgcggccgccctgtgacccaaacccgcagggcagcaggcacgatggacaggcccgcacagcggcctgagatccccaggacgcagcaccgctgtcaataggggccccaaatgcctggaccagggcctgcgtgggaaaggtctctggccacactcgggctttttgtgaagggccctcctgctgtgtgactacagtaactaccatagtgatgaacccagtggcaaaaactggctggaaacccaggggctgtgtgcacgcctcagcttggagctctccaggagcacaagagccgggcccaaggatttgtgcccagaccctcagcctctaggccccacgtccccagtcctgggggcccctggctcagctgtctggaccctccctgttccctgggaagctcctcctgacagccccgcctccagttccaggtgtggttattgtcaggcgatgtcagactgtggtggatatagtggctacgattaccacagtggtgccgcccatagcagcaaccaggccaagtagacaggcccctgctgcgcagccccaggcatccacttcacctgcttctcctggggctctcaaggctgctgtctgtcctctggccctctgtggcaggccccccagaaccagggttgagggacgccccgtcaaagccagacaaaaccaaggggtgttgagcccagcaagggaaggcccccaaacagaccaggaggtttctgaaggtgtctgtgtcacagtggggtatagcagcagctggtaccacagtgacactcacccagccagaaaccccattccaagtcagcggaagcagagagagcagggaggacacgtttaggatctgagactgcacctgacacccaggccagcagacgtctcccctccagggcaccccacacctaaaatgagccacagcctccggagcccccgcaggagaccccgcccacaagcccagcccccacccaggaggccccagagctcagggcgccccgtcggattccgaacagccccgagtcacagcgggtataaccggaaccaccactgtcagaatagctacgtcaaaaactgtccagtggccactgccggaggccccgccagagagggcagcagccactctgatcccatgtcctgccggctcccatgacccccagcacgcggagccccacaccctgagtttcagacaacaacccgctggaatgcacagtctcagcaggagaacagaccaaagccagcaaaagggacctcggtgacaccagtagggacaggaggattttgtgggggctcgtgtcactgtgaggatattgtagtggtggtagctgctactcccacagtgacacagacccattcccaaagccctactgcaaacacacccactcctggggctgaggggctgggggagcgtctgggaagtagggtccaggggtgtctatcaatgtccaaaatgcaccagactgcagtagacctgagagcgctgggcccacagcctcccctcggtgccctgctgcctcctcaggtcagccctggacatcccgggtttccccaggccagatggtaggtttgaagtgaggtctgtgtcactgtggtattatgattacgtttgggggagttatcgttatacccacagcatcacacggtccatcagaaacccatgccacagccctccccgcaggggaccgccgcgtgccatgttacgattttgatcgaggacacagcgccatgggtatggtggctaccacagcagtgcagcgaaaggcctgagatccccaggacgcagcaccactgtcaatgggggccccagacgcctggaccagggcctgcgtgggaaaggccgctgggcacactcaggggctttttgtgaaggcccctcctactgtgtgactacggtgactaccacagtgatgaaactagcagcaaaaactggccggacacccagggaccatgcacacttctcagcttggagctctccaggaccagaagagtcaggtctgagggtttgtagccagaccctcggcctctaggccccacgtccccagtcctgggggcccctggcacagctgtctggaccctccctcttccctgggaagctcctcctgacagccccgcctccagttccaggtgtggttattgtcagggggtgtcagactgtggtggatacagctatggttaccacagtggtgctgcccatagcagcaaccaggccaagtagacaggcccctgctgtgcagccccaggcctccagctcacctgcttctcctggggctctcaaggtcactgttgtctgtactctgccctctgggcaggccccccaaaaccagggttgagggatgatccgtcaaggcagacaagaccaaggggcactgaccccagcaagggaaggctcccaaacagacgaggaggtttctgaagctgtctgtatcacagtggggtatagcagtggctggtaccacagtgacactcgccaggccagaaaccccgtcccaagtcagcggaagcagagagagcagggaggacacgtttaggatctgaggccgcacctgacacccagggcagcagacgtctcccctccagggcataaagcgagccccagcctccagagccccctaagcattccccgcccagcagcccagcccctgcccccacccaggaggccccagagctcagggcgcctggtcggattctgaacagccccgagtcacagtgggtataactggaacgaccaccgtgagaaaaactgtgtccaaaactgactcctggcagcagtcggaggccccgccagagaggggagcagccggcctgaacccatgtcctgccggttcccatgacccccagcacccagagccccacgttcagacaacaacccgctggaatgcacagtctcagcaggagagccaggccagagccagcaagaggagactcggtgacaccagtctcctgtagggacaggaggattttgtgggggttcgtgtcactgtgagcatattgtggtggtgactgctattcccacagtgacacaaccccattcctaaagccctactgcaaacgcacccactcctgggactgaggggctgggggagcatctgggaagtatggcctaggggtgtccatcaatgcccaaaatgcaccagactccagtagacctgagagcgctgggcccacagcctcccctcggggccctgctgcctcctcaggtcagccctggacatcccgggtttccccaggcctggcggtaggtttgaagtgaggtctgtgtcactgtggtattactatgatagtagtggttattactaccacagtgtcacagagtccatcaaaaactcatgcctgggagcctcccaccacagccctccctgcgggggaccgctgcatgccgtgttaggattttgatcgaggacacggcgccatgggtatggtggctagaattcacgcgtagggtgagtcagacccacctgccctcaatggcaggcggggaagattcagaaaggcctgagatccccaggacgcagcaccactgtcaatgggggccccagacgcctggaccagggcctgtgtgggaaaggcctctggccacactcaggggctttttgtgaagggccctcctgctgtgtgactacggtggtaactcccacagtgatgaaaccagcagcaaaaactgaccggactcgcagggtttatgcacacttctcggctcggagctctccaggagcacaagagccaggcccgagggtttgtgcccagaccctcggcctctaggcccaggctctctagcactgggggcccctggcacagctgtctggaccctccctgttccctgggaagctcctcctgacagccccgcctccagttccaggtgtggttattgtcagggggtgccaggccgtggtagagatggctacaattaccacagtggtgccgcccatagcagcaaccaggccaagtagacagacccctgccacgcagccccaggcctccagctcacctgcttctcctggggctctcaaggctgctgtctgccctctggccctctgtgggccccccagaaccagtgttgagggacacccctgtccagggcagccaagtccaagaggcgcgctgagcccagcaagggaaggcccccaaacaaaccaggaggtttctgaagctgtctgtgtcacagtcgggtatagcagcggctaccacaatgacactgggcaggacagaaaccccatcccaagtcagccgaaggcagagagagcaggcaggacacatttaggatctgaggccacacctgacactcaagccaacagatgtctcccctccagggccacacctaaggtgagccacagccgccagagcctccacaggagaccccacgcagcagcccagcccctacccaggaggccccagagctcagggcgcctgggtggattctgaacagccccgagtcacggtgggtatagtgggagctactaccactgtgagaaaagctatgtccaaaactgtctcccggccactgctggaggcccagccagagaagggaccagccgcccgaacatacgaccttcccagccctcatgacccccagcacttggagctccacagtgtccccattggatggtgaggacgggggccggggccatctgcacctcccaacatcacccccaggcagcacaggcacaaaccccaaatccagagccgacaccaggaacacagacaccccaataccctgggggaccctggccctggtgacttcccactgggatccacccccgtgtccacctggatcaaagaccccaccgctgtctctgtccctcactcagggcctgctgaggggcgggtgctttggagcagactcaggtttaggggccaccattgtggggcccaacctcgaccaggacacagatttttctttcctgccctggggcaacacagactttggggtctgtgcagggaggaccttctggaaagtcaccaagcacagagccctgactgaggtggtctcaggaagacccccaggagggggtttgtgccccttcctctcatgtggaccccatgccccccaagataggggcatcatgcagggcaggtcctccatgcagccaccactaggcaactccctggcgccggtccccactgcgcctccatcccggctctggggatgcagccaccatggccacaccaggcagcccgggtccagcaaccctgcagtgcccaagcccttggcaggattcccagaggctggagcccacccctcctcatccccccacacctgcacacacacacctaccccctgcccagtccccctccaggagggttggagccgcccatagggtgggcgctccaggtctcactcactcgcttcccttcctgggcaaaggagcctcgtgccccggtcccccctgacggcgctgggcacaggtgtgggtactgggccccagggctcctccagccccagctgccctgctctccctgggaggcctgggcaccaccagaccaccagtccagggcacagccccagggagccgcccactgccagctcacaggaagaagataagcttcagaccctcagggccgggagctgccttcctgccaccccttcctgccccagacctccatgccctcccccaaccacttacacacaagccagggagctgtttccacacagttcaaccccaaaccaggacggcctggcactcgggtcactgccatttctgtctgcattcgctcccagcgcccctgtgttccctccctcctccctccttcctttcttcctgcattgggttc

SEQ ID NO: 2 - DNA, 8841 bp, synthetic construct
  misc_feature 1..8841: note = nucleotide sequence of human minimized D region with substitutedbovine ORFs
  misc_feature 737..767: note = B1-1 substituted for D2-2
  misc_feature 1024..1039: note = B2-1 substituted for D3-3
  misc_feature 1296..1331: note = B3-1 substituted for D4-4
  misc_feature 1588..1630: note = B4-1 substituted for D5-5
  misc_feature 1887..1900: note = B9-1 substituted for D6-6
  misc_feature 2157..2187: note = B1-2 substituted for D1-7
  misc_feature 2444..2459: note = B2-2 substituted for D2-8
  misc_feature 2715..2756: note = B5-2 substituted for D3-9
  misc_feature 2910..3057: note = B8-2 substituted for D3-10
  misc_feature 3374..3431: note = B6-2 substituted for D4-11
  misc_feature 3688..3806: note = B1-3 substituted for D5-12
  misc_feature 4063..4078: note = B2-3 substituted for D6-13
  misc_feature 4338..4373: note = B3-3 substituted for D1-14
  misc_feature 4630..4696: note = B7-3 substituted for D2-15
  misc_feature 4953..4994: note = B5-3 substituted for D3-16
  misc_feature 5251..5308: note = B6-3 substituted for D4-17
  misc_feature 5565..5595: note = B1-4 substituted for D5-18
  misc_feature 5852..5867: note = B2-4 substituted for D6-19
  misc_feature 6124..6159: note = B3-4 substituted for D1-20
  misc_feature 6416..6488: note = B7-4 substituted for D1-21
  misc_feature 6745..6785: note = B5-4 substituted for D3-22
  misc_feature 7103..7160: note = B6-4 substituted for D4-23
  misc_feature 7417..7430: note = B9-4 substituted for D5-24
  source 1..8841: mol_type = other DNA
gtcgcctctacgggaaatccgggactcagcagtaaccctcaggaagcagggcccaggcgccgtttaataggaggcttcctcacaatgaaacttttagaaagccttgactacaatgatgaccttggtgtggctgtgaacactgtcagctcccacagctgctgcagcaaaaaatgtccatagacagggtgggggcccggggtcgtctgctgtcctgctcagcccacagcacgcatggaggatctgaggtgccacacctgacgcccaggccagaacatgcctccctccagggtgacctgccatgtcctgcattgctggagggacaggggcagcctatgaggatctggggccaggagatgaatcctattaacccagaggaaaactaacaggacccaagcaccctccccgttgaagctgacctgcccagaggggcctgggcccaccccacacaccggggcggaatgtgtacaggccccggtctctgtgggtgttccgctaactggggctcccagtgctcaccccacaactaaagcgagccccagcctccagagcccccgaaggagatgccgcccacaagcccagcccccatccaggaggccccagagctcaggccctgagtttcagacaaaaaccccctggaaatcatagtatcagcaggagaactagccagagacagcaagaggggactcagtgactcccgcggggacaggaggattttgtgggggctcgtgtcactgtgagaataccgtgatgatggttactgctacacccacagtgacacagccccattcccaaagccctgctgtaaacgcttccacttctggagctgaggggctggggggagcgtctgggaagtagggcctaggggtggccatcaatgcccaaaacgcaccagactcagtagacctgagagcgctgggcccacagcctcccctcggtgccctgctacctcctcaggtcagccctggacatcccgggtttccccaggcctggcggtaggtttggggtgaggtctgtgtcactgtgttactatagtgaccaccacagtgtcacagagtccatcaaaaacccatccctgggaaccttctgccacagccctccctgtggggcaccgctgcgtgccatgttaggattttgactgaggacacagcaccatgggtatggtggctagaaaggtctgagatccccaggacgcagcaccactgtcaatgggggccccagacgcctggaccagggcctgcgtgggaaaggcctctgggcacactcaggggctttttgtgaagggtcctcctactgtggtattgtggtagctattgtggtagttattatggtaccacagtgatgaacccagcagcaaaaactgaccggactcccaaggtttatgcacacttctccgctcagagctctccaggatcagaagagccgggcccaagggtttctgcccagaccctcggcctctaggccccatgtccccagtcctgggggcccctggcacagctgtctggaccctctctattccctgggaagctcctcctgacagccccgcctccagttccaggtgtggttattgtcagggggtgtcagactgtggtagttatagtggttatggttatggttatagttatggttataccacagtggtgctgcccatagcagcaaccaggccaagtagacaggcccctgctgtgcagccccaggcctccagctcacctgcttctcctggggctctcaaggctgctgttttctgcactctcccctctgggcaggccccccagaaccagggatgaggacgccccgtcaaggccagaaaagaccaagttgtgctgagcccagcaagggaaggtccccaaacaaaccaggaagtttctgaaggtgtctgtgtcacagtggaactcggtggggccacagtgacactcgccaggccagaaaccccatcccaagtcagcggaatgcagagagagcagggaggacatgtttaggatctgaggccgcacctgacacccaggccagcagacgtctcctgtccatggcccacacctaaaacgagccacagcctcagagcccctgaaggagaccccgcccacaagcccagcccccacccaggaggccccagagcacagggcgccccgtcggattctgaacagccccgagtcacagtgagaatatcgtgatgatggttactgctacacccactgtgagaaaagcttcgtccaaaacggtctcctggccacagtcggaggccccgccagagaggggagcagccaccccaaacccatgttctgccggctcccatgaccccgtgcacctggagccccacacccagagtttcagacaaaaaccccctggaatgcacagtctcagcaggagagccagccagagccagcaagatggggctcagtgacacccgcagggacaggaggattttgtgggggctcgtgtcactgtgttactatagtgaccaccacagtgacacagccccattcccaaagccctactgcaaacgcattccacttctggggctgaggggctgggggagcgtctgggaaatagggctcaggggtgtccatcaatgcccaaaacgcaccagaccagcagacctgagagcgctgggcccacagcctcccctcagagccctgctgcctcctccggtcagccctggacatcccaggtttccccaggcctgccggtaggtttagaatgaggtctgtgtcactgtgatgatacgataggtgtggttgtagttattgtagtgttgctaccacagtgtcacagagtccatcaaaaacccatgcctggaagcttcccgccacagccctccccatggggccctgctgcctcctcaggtcagccccggacatcccgggtttccccaggctgggcggtaggtttggggtgaggtctgtgtcactgtggtagttgtcctgatggttatagttatggttatggttgtggttatggttatggttgtagtggttatgattgttatggttatggtggttatggtggttatggtggttatggttatagtagttatagttatagttatacttacgaatataccacagtgtcacagagtccatcaaaaacccatccctgggagcctcccgccacagccctccctgcaggggaccggtacgtgccatgttaggattttgatcgaggagacagcaccatgggtatggtggctaatgcatgcggccgccctgtgacccaaacccgcagggcagcaggcacgatggacaggcccgcacagcggcctgagatccccaggacgcagcaccgctgtcaataggggccccaaatgcctggaccagggcctgcgtgggaaaggtctctggccacactcgggctttttgtgaagggccctcccacagtggtagttgttatagtggttatggttatggttgtggttatggttatggttatgattataccatagtgatgaacccagtggcaaaaactggctggaaacccaggggctgtgtgcacgcctcagcttggagctctccaggagcacaagagccgggcccaaggatttgtgcccagaccctcagcctctaggccccacgtccccagtcctgggggcccctggctcagctgtctggaccctccctgttccctgggaagctcctcctgacagccccgcctccagttccaggtgtggttattgtcaggcgatgtcagactgtgagactatcgtgatgatggttactgctacacccacagtgactcaggccctgacataaagtctgacccgcacacaggtgtggagctggccaatgcatccccaggggcactgggctcccaagcacagtggtgccgcccatagcagcaaccaggccaagtagacaggcccctgctgcgcagccccaggcatccacttcacctgcttctcctggggctctcaaggctgctgtctgtcctctggccctctgtggcaggccccccagaaccagggttgagggacgccccgtcaaagccagacaaaaccaaggggtgttgagcccagcaagggaaggcccccaaacagaccaggaggtttctgaaggtgtctgtgtcacagtgttactatagtgaccaccacagtgacactcacccagccagaaaccccattccaagtcagcggaagcagagagagcagggaggacacgtttaggatctgagactgcacctgacacccaggccagcagacgtctcccctccagggcaccccacacctaaaatgagccacagcctccggagcccccgcaggagaccccgcccacaagcccagcccccacccaggaggccccagagctcagggcgccccgtcggattccgaacagccccgagtcacagtggtattgtggtagctattgtggtagttattatggtaccactgtcagaatagctacgtcaaaaactgtccagtggccactgccggaggccccgccagagagggcagcagccactctgatcccatgtcctgccggctcccatgacccccagcacgcggagccccacaccctgagtttcagacaacaacccgctggaatgcacagtctcagcaggagaacagaccaaagccagcaaaagggacctcggtgacaccagtagggacaggaggattttgtgggggctcgtgtcactgtggtagttatggtggttatggttatggtggttatggttgttatggttatggttatggttatggttataccacagtgacacagacccattcccaaagccctactgcaaacacacccactcctggggctgaggggctgggggagcgtctgggaagtagggtccaggggtgtctatcaatgtccaaaatgcaccagactgcagtagacctgagagcgctgggcccacagcctcccctcggtgccctgctgcctcctcaggtcagccctggacatcccgggtttccccaggccagatggtaggtttgaagtgaggtctgtgtcactgtgatgatacgataggtgtggttttagttattgtagtgttgctaccacagcatcacacggtccatcagaaacccatgccacagccctccccgcaggggaccgccgcgtgccatgttacgattttgatcgaggacacagcgccatgggtatggtggctaccacagcagtgcagcgaaaggcctgagatccccaggacgcagcaccactgtcaatgggggccccagacgcctggaccagggcctgcgtgggaaaggccgctgggcacactcaggggctttttgtgaaggcccctcctactgtggtagttgttatagtggttatggttatggttatggttgtggttatggttatggttataccacagtgatgaaactagcagcaaaaactggccggacacccagggaccatgcacacttctcagcttggagctctccaggaccagaagagtcaggtctgagggtttgtagccagaccctcggcctctaggccccacgtccccagtcctgggggcccctggcacagctgtctggaccctccctcttccctgggaagctcctcctgacagccccgcctccagttccaggtgtggttattgtcagggggtgtcagactgtgagaatatcgtgatgatggttactgctacacccacagtggtgctgcccatagcagcaaccaggccaagtagacaggcccctgctgtgcagccccaggcctccagctcacctgcttctcctggggctctcaaggtcactgttgtctgtactctgccctctgggcaggccccccaaaaccagggttgagggatgatccgtcaaggcagacaagaccaaggggcactgaccccagcaagggaaggctcccaaacagacgaggaggtttctgaagctgtctgtatcacagtgttactatagtgaccaccacagtgacactcgccaggccagaaaccccgtcccaagtcagcggaagcagagagagcagggaggacacgtttaggatctgaggccgcacctgacacccagggcagcagacgtctcccctccagggcataaagcgagccccagcctccagagccccctaagcattccccgcccagcagcccagcccctgcccccacccaggaggccccagagctcagggcgcctggtcggattctgaacagccccgagtcacagtggtattgtggtagctattgtggtagttattatggtaccaccgtgagaaaaactgtgtccaaaactgactcctggcagcagtcggaggccccgccagagaggggagcagccggcctgaacccatgtcctgccggttcccatgacccccagcacccagagccccacgttcagacaacaacccgctggaatgcacagtctcagcaggagagccaggccagagccagcaagaggagactcggtgacaccagtctcctgtagggacaggaggattttgtgggggttcgtgtcactgtggtagttatggtggttatggttatggtggttatggttgttatggttatggttatggttatggttatggttataccacagtgacacaaccccattcctaaagccctactgcaaacgcacccactcctgggactgaggggctgggggagcatctgggaagtatggcctaggggtgtccatcaatgcccaaaatgcaccagactccagtagacctgagagcgctgggcccacagcctcccctcggggccctgctgcctcctcaggtcagccctggacatcccgggtttccccaggcctggcggtaggtttgaagtgaggtctgtgtcactgtgatgatacgataggtgtggttttagttattgtagtgttgctaccacagtgtcacagagtccatcaaaaactcatgcctgggagcctcccaccacagccctccctgcgggggaccgctgcatgccgtgttaggattttgatcgaggacacggcgccatgggtatggtggctagaattcacgcgtagggtgagtcagacccacctgccctcaatggcaggcggggaagattcagaaaggcctgagatccccaggacgcagcaccactgtcaatgggggccccagacgcctggaccagggcctgtgtgggaaaggcctctggccacactcaggggctttttgtgaagggccctcccacagtggtagttgttatagtggttatggttatggttatggttgtggttatggttatggttataccacagtgatgaaaccagcagcaaaaactgaccggactcgcagggtttatgcacacttctcggctcggagctctccaggagcacaagagccaggcccgagggtttgtgcccagaccctcggcctctaggcccaggctctctagcactgggggcccctggcacagctgtctggaccctccctgttccctgggaagctcctcctgacagccccgcctccagttccaggtgtggttattgtcagggggtgccacacagtggaactcggtggggccacagtggtgccgcccatagcagcaaccaggccaagtagacagacccctgccacgcagccccaggcctccagctcacctgcttctcctggggctctcaaggctgctgtctgccctctggccctctgtggtctcccggccactgctggaggcccagccagagaagggaccagccgcccgaacatacgaccttcccagccctcatgacccccagcacttggagctccacagtgtccccattggatggtgaggacgggggccggggccatctgcacctcccaacatcacccccaggcagcacaggcacaaaccccaaatccagagccgacaccaggaacacagacaccccaataccctgggggaccctggccctggtgacttcccactgggatccacccccgtgtccacctggatcaaagaccccaccgctgtctctgtccctcactcagggcctgctgaggggcgggtgctttggagcagactcaggtttaggggccaccattgtggggcccaacctcgaccaggacacagatttttctttcctgccctggggcaacacagactttggggtctgtgcagggaggaccttctggaaagtcaccaagcacagagccctgactgaggtggtctcaggaagacccccaggagggggtttgtgccccttcctctcatgtggaccccatgccccccaagataggggcatcatgcagggcaggtcctccatgcagccaccactaggcaactccctggcgccggtccccactgcgcctccatcccggctctggggatgcagccaccatggccacaccaggcagcccgggtccagcaaccctgcagtgcccaagcccttggcaggattcccagaggctggagcccacccctcctcatccccccacacctgcacacacacacctaccccctgcccagtccccctccaggagggttggagccgcccatagggtgggcgctccaggtctcactcactcgcttcccttcctgggcaaaggagcctcgtgccccggtcccccctgacggcgctgggcacaggtgtgggtactgggccccagggctcctccagccccagctgccctgctctccctgggaggcctgggcaccaccagaccaccagtccagggcacagccccagggagccgcccactgccagctcacaggaagaagataagcttcagaccctcagggccgggagctgccttcctgccaccccttcctgccccagacctccatgccctcccccaaccacttacacacaagccagggagctgtttccacacagttcaaccccaaaccaggacggcctggcactcgggtcactgccatttctgtctgcattcgctcccagcgcccctgtgttccctccctcctccctccttcctttcttcctgcattgggttc

SEQ ID NO: 3 - DNA, 9889 bp, synthetic construct
  misc_feature 1..9889: note = nucleotide sequence of human minimized D region with modifiedORFs
  misc_feature 647..690: note = modified D1-1
  misc_feature 947..990: note = modified D2-2
  misc_feature 1247..1290: note = modified D3-3
  misc_feature 1547..1590: note = modified D4-4
  misc_feature 1847..1890: note = modified D5-5
  misc_feature 2147..2190: note = modified D6-6
  misc_feature 2447..2508: note = modified D1-7
  misc_feature 2765..2808: note = modified DL2-8
  misc_feature 3064..3149: note = modified D3-9
  misc_feature 3303..3385: note = modified D3-10
  misc_feature 3702..3760: note = modified D4-11
  misc_feature 4017..4078: note = modified D5-12
  misc_feature 4335..4384: note = modified D6-13
  misc_feature 4644..4711: note = modified D1-14
  misc_feature 4968..5035: note = modified D2-15
  misc_feature 5292..5365: note = modified D3-16
  misc_feature 5622..5695: note = modified D4-17
  misc_feature 5952..6016: note = modified D5-18
  misc_feature 6273..6334: note = modified D6-19
  misc_feature 6591..6652: note = modified D1-20
  misc_feature 6909..6961: note = modified D2-21
  misc_feature 7218..7264: note = modified D3-22
  misc_feature 7581..7642: note = modified D4-23
  misc_feature 7899..7960: note = modified D5-24
  misc_feature 8217..8263: note = modified D6-25
  misc_feature 8520..8578: note = modified D1-26
  source 1..9889: mol_type = other DNA
gtcgcctctacgggaaatccgggactcagcagtaaccctcaggaagcagggcccaggcgccgtttaataggaggcttcctcacaatgaaacttttagaaagccttgactacaatgatgaccttggtgtggctgtgaacactgtcagctcccacagctgctgcagcaaaaaatgtccatagacagggtgggggcccggggtcgtctgctgtcctgctcagcccacagcacgcatggaggatctgaggtgccacacctgacgcccaggccagaacatgcctccctccagggtgacctgccatgtcctgcattgctggagggacaggggcagcctatgaggatctggggccaggagatgaatcctattaacccagaggaaaactaacaggacccaagcaccctccccgttgaagctgacctgcccagaggggcctgggcccaccccacacaccggggcggaatgtgtacaggccccggtctctgtgggtgttccgctaactggggctcccagtgctcaccccacaactaaagcgagccccagcctccagagcccccgaaggagatgccgcccacaagcccagcccccatccaggaggccccagagctcagggcgccggggcagattctgaacagccccgagtcacggtggggcacaactggatggggctggctgggcaaacctatcggagcttcaccgtgagaaaaactgtgtccaaaactctctcctggcccctgctggaggccgcgccagagaggggagcagccgccccgaacctaggtcctgctcagctcacacgacccccagcagccagagcacagtccctgagtttcagacaaaaaccccctggaaatcatagtatcagcaggagaactagccagagacagcaagaggggactcagtgactcccgcggggacaggaggattttgtgggggctcgtgtcactgtgcggcaggaatggctgggatattgtagccaccacaagcacccagtcacagtgacacagccccattcccaaagccctgctgtaaacgcttccacttctggagctgaggggctggggggagcgtctgggaagtagggcctaggggtggccatcaatgcccaaaacgcaccagactcagtagacctgagagcgctgggcccacagcctcccctcggtgccctgctacctcctcaggtcagccctggacatcccgggtttccccaggcctggcggtaggtttggggtgaggtctgtgtcactgtggtgtatcacaatctttggagtggtgatccctcagagcggcccctcacagtgtcacagagtccatcaaaaacccatccctgggaaccttctgccacagccctccctgtggggcaccgctgcgtgccatgttaggattttgactgaggacacagcaccatgggtatggtggctagaaaggtctgagatccccaggacgcagcaccactgtcaatgggggccccagacgcctggaccagggcctgcgtgggaaaggcctctgggcacactcaggggctttttgtgaagggtcctcctactgtggcctgcagcagcttggttcagtgtatttaagcccccactcaattcacagtgatgaacccagcagcaaaaactgaccggactcccaaggtttatgcacacttctccgctcagagctctccaggatcagaagagccgggcccaagggtttctgcccagaccctcggcctctaggccccatgtccccagtcctgggggcccctggcacagctgtctggaccctctctattccctgggaagctcctcctgacagccccgcctccagttccaggtgtggttattgtcagggggtgtcagactgtggggcgatgacagcagcggctacagcatcaccgccatcgagtattcacagtggtgctgcccatagcagcaaccaggccaagtagacaggcccctgctgtgcagccccaggcctccagctcacctgcttctcctggggctctcaaggctgctgttttctgcactctcccctctgggcaggccccccagaaccagggatgaggacgccccgtcaaggccagaaaagaccaagttgtgctgagcccagcaagggaaggtccccaaacaaaccaggaagtttctgaaggtgtctgtgtcacagtgaggcccatacagctgggacgacagcccccaggacaattactatacacagtgacactcgccaggccagaaaccccatcccaagtcagcggaatgcagagagagcagggaggacatgtttaggatctgaggccgcacctgacacccaggccagcagacgtctcctgtccatggcccacacctaaaacgagccacagcctcagagcccctgaaggagaccccgcccacaagcccagcccccacccaggaggccccagagcacagggcgccccgtcggattctgaacagccccgagtcacagtgactgcacggccggaggatctacggcattgttgcattcaatgagtggttcacctacttctacacactgtgagaaaagcttcgtccaaaacggtctcctggccacagtcggaggccccgccagagaggggagcagccaccccaaacccatgttctgccggctcccatgaccccgtgcacctggagccccacacccagagtttcagacaaaaaccccctggaatgcacagtctcagcaggagagccagccagagccagcaagatggggctcagtgacacccgcagggacaggaggattttgtgggggctcgtgtcactgtgcagacaccacgacgtgttcatgctggtaccaatcgccggctggtcacagtgacacagccccattcccaaagccctactgcaaacgcattccacttctggggctgaggggctgggggagcgtctgggaaatagggctcaggggtgtccatcaatgcccaaaacgcaccagaccagcagacctgagagcgctgggcccacagcctcccctcagagccctgctgcctcctccggtcagccctggacatcccaggtttccccaggcctgccggtaggtttagaatgaggtctgtgtcactgtgcagcaagcacagactgcgggactacgtgctgtacgacgactacgggctgatcaactatcaggagtggaacgactacctggagttcccacagtgtcacagagtccatcaaaaacccatgcctggaagcttcccgccacagccctccccatggggccctgctgcctcctcaggtcagccccggacatcccgggtttccccaggctgggcggtaggtttggggtgaggtctgtgtcactgtgaagcaagcaccgcctgagagattacttcctgtacaacgagtatggccccaactacgaggagtggggcgactatctggcaaccccacagtgtcacagagtccatcaaaaacccatccctgggagcctcccgccacagccctccctgcaggggaccggtacgtgccatgttaggattttgatcgaggagacagcaccatgggtatggtggctaatgcatgcggccgccctgtgacccaaacccgcagggcagcaggcacgatggacaggcccgcacagcggcctgagatccccaggacgcagcaccgctgtcaataggggccccaaatgcctggaccagggcctgcgtgggaaaggtctctggccacactcgggctttttgtgaagggccctcctgctgtgcaagtcttgttgtggcggcaggagatactgcaacggagctgactgcttcaactgggactcatagtgatgaacccagtggcaaaaactggctggaaacccaggggctgtgtgcacgcctcagcttggagctctccaggagcacaagagccgggcccaaggatttgtgcccagaccctcagcctctaggccccacgtccccagtcctgggggcccctggctcagctgtctggaccctccctgttccctgggaagctcctcctgacagccccgcctccagttccaggtgtggttattgtcaggcgatgtcagactgtgccagctgggctacgacttctggtccggctactacaccgacaccctgtactactatttcggcacacagtggtgccgcccatagcagcaaccaggccaagtagacaggcccctgctgcgcagccccaggcatccacttcacctgcttctcctggggctctcaaggctgctgtctgtcctctggccctctgtggcaggccccccagaaccagggttgagggacgccccgtcaaagccagacaaaaccaaggggtgttgagcccagcaagggaaggcccccaaacagaccaggaggtttctgaaggtgtctgtgtcacagtgcggcaagtactacgacttctggagcggctatcctcctggcgaggagtactcacagtgacactcacccagccagaaaccccattccaagtcagcggaagcagagagagcagggaggacacgtttaggatctgagactgcacctgacacccaggccagcagacgtctcccctccagggcaccccacacctaaaatgagccacagcctccggagcccccgcaggagaccccgcccacaagcccagcccccacccaggaggccccagagctcagggcgccccgtcggattccgaacagccccgagtcacagcggttccaggagagcggccctcctagactggatagatggtccggcaggaactactactactacagcggcacactgtcagaatagctacgtcaaaaactgtccagtggccactgccggaggccccgccagagagggcagcagccactctgatcccatgtcctgccggctcccatgacccccagcacgcggagccccacaccctgagtttcagacaacaacccgctggaatgcacagtctcagcaggagaacagaccaaagccagcaaaagggacctcggtgacaccagtagggacaggaggattttgtgggggctcgtgtcactgtgtggcgaggagcacgaggtaccacagctgcactcctggagcggcagaaatctgtaccactatacaggcgcacagtgacacagacccattcccaaagccctactgcaaacacacccactcctggggctgaggggctgggggagcgtctgggaagtagggtccaggggtgtctatcaatgtccaaaatgcaccagactgcagtagacctgagagcgctgggcccacagcctcccctcggtgccctgctgcctcctcaggtcagccctggacatcccgggtttccccaggccagatggtaggtttgaagtgaggtctgtgtcactgtgagcaggcggccctgactacaggaacggctacaactactacgacttttacgatggctactacaactaccactacacacagcatcacacggtccatcagaaacccatgccacagccctccccgcaggggaccgccgcgtgccatgttacgattttgatcgaggacacagcgccatgggtatggtggctaccacagcagtgcagcgaaaggcctgagatccccaggacgcagcaccactgtcaatgggggccccagacgcctggaccagggcctgcgtgggaaaggccgctgggcacactcaggggctttttgtgaaggcccctcctactgtgggcaggcggccccatctggcacgacgacgtgaagtactacgactttaacgatggctattacaattaccactacacacagtgatgaaactagcagcaaaaactggccggacacccagggaccatgcacacttctcagcttggagctctccaggaccagaagagtcaggtctgagggtttgtagccagaccctcggcctctaggccccacgtccccagtcctgggggcccctggcacagctgtctggaccctccctcttccctgggaagctcctcctgacagccccgcctccagttccaggtgtggttattgtcagggggtgtcagactgtgtataccccccccttcggtattacggtattttgactggttaccccccagggagggttactacggtacacagtggtgctgcccatagcagcaaccaggccaagtagacaggcccctgctgtgcagccccaggcctccagctcacctgcttctcctggggctctcaaggtcactgttgtctgtactctgccctctgggcaggccccccaaaaccagggttgagggatgatccgtcaaggcagacaagaccaaggggcactgaccccagcaagggaaggctcccaaacagacgaggaggtttctgaagctgtctgtatcacagtgcaccgactacaccatcgacgatgccggcatccactatcagggctctggcacattctggtactcacagtgacactcgccaggccagaaaccccgtcccaagtcagcggaagcagagagagcagggaggacacgtttaggatctgaggccgcacctgacacccagggcagcagacgtctcccctccagggcataaagcgagccccagcctccagagccccctaagcattccccgcccagcagcccagcccctgcccccacccaggaggccccagagctcagggcgcctggtcggattctgaacagccccgagtcacagtgcaccgactacaccatcgacgatcagggaaggttctaccagggcagcggcaccttctggtattcaccgtgagaaaaactgtgtccaaaactgactcctggcagcagtcggaggccccgccagagaggggagcagccggcctgaacccatgtcctgccggttcccatgacccccagcacccagagccccacgttcagacaacaacccgctggaatgcacagtctcagcaggagagccaggccagagccagcaagaggagactcggtgacaccagtctcctgtagggacaggaggattttgtgggggttcgtgtcactgtggaaccactacggctctggcagctacttttataggacagcctactactacgccacacagtgacacaaccccattcctaaagccctactgcaaacgcacccactcctgggactgaggggctgggggagcatctgggaagtatggcctaggggtgtccatcaatgcccaaaatgcaccagactccagtagacctgagagcgctgggcccacagcctcccctcggggccctgctgcctcctcaggtcagccctggacatcccgggtttccccaggcctggcggtaggtttgaagtgaggtctgtgtcactgtgtattaggcggggaggaggggctcgctattactatcatgaggcaggggcacagtgtcacagagtccatcaaaaactcatgcctgggagcctcccaccacagccctccctgcgggggaccgctgcatgccgtgttaggattttgatcgaggacacggcgccatgggtatggtggctagaattcacgcgtagggtgagtcagacccacctgccctcaatggcaggcggggaagattcagaaaggcctgagatccccaggacgcagcaccactgtcaatgggggccccagacgcctggaccagggcctgtgtgggaaaggcctctggccacactcaggggctttttgtgaagggccctcctgctgtgcaagcacggcaggcgcatctatggcgtggttgcctttaaggagtggttcacctacttttacacacagtgatgaaaccagcagcaaaaactgaccggactcgcagggtttatgcacacttctcggctcggagctctccaggagcacaagagccaggcccgagggtttgtgcccagaccctcggcctctaggcccaggctctctagcactgggggcccctggcacagctgtctggaccctccctgttccctgggaagctcctcctgacagccccgcctccagttccaggtgtggttattgtcagggggtgccaggccgtgcctgcacggcaagcgcatctatggcattgtggccctgggcgagctgttcacctacttttacacacagtggtgccgcccatagcagcaaccaggccaagtagacagacccctgccacgcagccccaggcctccagctcacctgcttctcctggggctctcaaggctgctgtctgccctctggccctctgtgggccccccagaaccagtgttgagggacacccctgtccagggcagccaagtccaagaggcgcgctgagcccagcaagggaaggcccccaaacaaaccaggaggtttctgaagctgtctgtgtcacagtccatgagacctgttgaccacggcatcgactacagcgggctgttcgtgtcacaatgacactgggcaggacagaaaccccatcccaagtcagccgaaggcagagagagcaggcaggacacatttaggatctgaggccacacctgacactcaagccaacagatgtctcccctccagggccacacctaaggtgagccacagccgccagagcctccacaggagaccccacgcagcagcccagcccctacccaggaggccccagagctcagggcgcctgggtggattctgaacagccccgagtcacggtgagggcaaggtgatagcagcagctggtacccccagggtttttactactactactacggtacactgtgagaaaagctatgtccaaaactgtctcccggccactgctggaggcccagccagagaagggaccagccgcccgaacatacgaccttcccagccctcatgacccccagcacttggagctccacagtgtccccattggatggtgaggacgggggccggggccatctgcacctcccaacatcacccccaggcagcacaggcacaaaccccaaatccagagccgacaccaggaacacagacaccccaataccctgggggaccctggccctggtgacttcccactgggatccacccccgtgtccacctggatcaaagaccccaccgctgtctctgtccctcactcagggcctgctgaggggcgggtgctttggagcagactcaggtttaggggccaccattgtggggcccaacctcgaccaggacacagatttttctttcctgccctggggcaacacagactttggggtctgtgcagggaggaccttctggaaagtcaccaagcacagagccctgactgaggtggtctcaggaagacccccaggagggggtttgtgccccttcctctcatgtggaccccatgccccccaagataggggcatcatgcagggcaggtcctccatgcagccaccactaggcaactccctggcgccggtccccactgcgcctccatcccggctctggggatgcagccaccatggccacaccaggcagcccgggtccagcaaccctgcagtgcccaagcccttggcaggattcccagaggctggagcccacccctcctcatccccccacacctgcacacacacacctaccccctgcccagtccccctccaggagggttggagccgcccatagggtgggcgctccaggtctcactcactcgcttcccttcctgggcaaaggagcctcgtgccccggtcccccctgacggcgctgggcacaggtgtgggtactgggccccagggctcctccagccccagctgccctgctctccctgggaggcctgggcaccaccagaccaccagtccagggcacagccccagggagccgcccactgccagctcacaggaagaagataagcttcagaccctcagggccgggagctgccttcctgccaccccttcctgccccagacctccatgccctcccccaaccacttacacacaagccagggagctgtttccacacagttcaaccccaaaccaggacggcctggcactcgggtcactgccatttctgtctgcattcgctcccagcgcccctgtgttccctccctcctccctccttcctttcttcctgcattgggttc

SEQ ID NO: 4 - DNA, 23 bp, synthetic construct
  misc_feature 1..23: note = target nucleotide sequence of gRNA Up3
  misc_feature 21..23: note = PAM sequence
  source 1..23: mol_type = other DNA
agatcctccatgcgtgctgtggg

SEQ ID NO: 5 - DNA, 23 bp, synthetic construct
  misc_feature 1..23: note = target nucleotide sequence of gRNA Down4
  misc_feature 21..23: note = PAM sequence
  source 1..23: mol_type = other DNA
ctgcggcatgaacccaatgcagg

SEQ ID NO: 6 - DNA, 28 bp, synthetic construct
  misc_feature 1..28: note = primer
  source 1..28: mol_type = other DNA
tcccacggcccaaggaagacaagacaca

SEQ ID NO: 7 - DNA, 28 bp, synthetic construct
  misc_feature 1..28: note = primer
  source 1..28: mol_type = other DNA
tcgaacacgctcctagcattgcacagcc

SEQ ID NO: 8 - DNA, 20 bp, synthetic construct
  misc_feature 1..20: note = primer
  source 1..20: mol_type = other DNA
acacctgtctccgggttgtg

SEQ ID NO: 9 - DNA, 20 bp, synthetic construct
  misc_feature 1..20: note = primer
  source 1..20: mol_type = other DNA
aagaaacgcaggacggtgga

SEQ ID NO: 10 - DNA, 20 bp, synthetic construct
  misc_feature 1..20: note = primer
  source 1..20: mol_type = other DNA
cagcagccactctgatccca

SEQ ID NO: 11 - DNA, 20 bp, synthetic construct
  misc_feature 1..20: note = primer
  source 1..20: mol_type = other DNA
ctggtggactctacggcgaa

SEQ ID NO: 12 - DNA, 20 bp, synthetic construct
  misc_feature 1..20: note = primer
  source 1..20: mol_type = other DNA
gggaccctcaaggtgtgaac

SEQ ID NO: 13 - DNA, 20 bp, synthetic construct
  misc_feature 1..20: note = primer
  source 1..20: mol_type = other DNA
agggtgcttgggtcctgtta

SEQ ID NO: 14 - DNA, 20 bp, synthetic construct
  misc_feature 1..20: note = primer
  source 1..20: mol_type = other DNA
acaagccagggagctgtttc

SEQ ID NO: 15 - DNA, 20 bp, synthetic construct
  misc_feature 1..20: note = primer
  source 1..20: mol_type = other DNA
tcaagaaatccgaggcgaca

SEQ ID NO: 16 - DNA, 959 bp, Homo sapiens
  source 1..959: mol_type = unassigned DNA
gacctgagagccgctccctgaagtgtccccattgggaaggatggggcctgtgtctccaggctctgggaggacagaatcctgacctcaacagtggccggcacggacacaactggccccatcccggggacgctgaccagcgctgggcaacttttcccttccccgacgactgagccccgagcaccctccctgctcccctaccacctccctttacaaggctgtggcctctgcacagatgataatggagcttggctcattcccctagagtcggtagggagttaaggacaaaactcagtttcctccacctgaactcaagtctgcctatgtttacctaatcacacctggtggacagtttggacaaacttgcacactcagagacacagacacttctagaaatcattatctccctgccccggggaccccactccagcagaagtctgctaggcactggcctgggccctcctgctgtcctaggaggctgctgacctcctgcctggctcctgtccccaggtccagagtcagagcagactccagggacgctgcaggctaggaagccgccccctccaggcgagggtctagtgcaggtgcccaggacaagaaagattgtgaatgcaggaatgactgggccacacccctcccgtgcacgccccctcctgccctgcaccccacagcccagccccccgtgctggatgcccccccacagcagaggtgctgttctgtgatcccctgggaaagacgccctcaacctccaccctgtcccacggcccaaggaagacaagacacaggccctctcctcacagtctccccacctggctcctgctgggaccctcaaggtgtgaacagggaggatggttgtctgggtggcccctaggagcccagatcttcactccacagaccccaacccaagcacccccttctgcagggcccagctcatccccctcctcctccctctgctctcctct

SEQ ID NO: 17 - DNA, 981 bp, Homo sapiens
  source 1..981: mol_type = unassigned DNA
ctcactgaaggcagcctcagggtgcccaggggcaggcagggtgggggtgaggcttccagctccaaccgctccactagccgagactaaggaagtgagaggcagccagaaatccagaccattccatagcaaatggatttcattaaagttaccagacttcagtgtaagtaacatgagccccatgcacaacaatcccttatgaaggggaagtcagtgtcgcctcggatttcttgaaaaacacaaaaacttatcaatgcctgtaaaagtctgttggaaagaaaatatgattcaagaatgttatgcccaacaaagctggcatattttctacccggacacactcagggaatgtggtcccttgagtgcttctctcactgcgtaaatcctacgtggtgtttaagcatattcataaatgtgtatgtctatttttatgtgtaagatggttcatttttattttatttattcaatatgtacaataaagaatattgacaaataggctggacatggtggctcccacctgtaatcccagccctttgggaggccgaggcgggcagatcacctgaggtctggagttcgagaccagcctggccaacatgatgaaaacccatctctactaaaaatacaaagattagccaggcatggtggtgcatgcctgtaatcccagccactcaggaggctgagacaggagaaatgcgtgaacccggaaggcggaggttgcagtgagccgagatcacaccactgcactccagcctggcgacagagcaagattccatctcaaaaaaaaaaagacaaagaaatttgtttttttgaataaagacaaatttcatcacacgaagataaagatgcaaagctccagacaggaaggcacggacagcacagtgaagcccggagcgggcgctggggggccaggggcatggcgggggtgccagcgtctctcggtgcctaccatggccactccagcctgtgttctcacgaggatggctgtgt

SEQ ID NO: 18 - DNA, 77 bp, synthetic construct
  misc_feature 1..77: note = nucleotide sequence of Bxb1 attB
  source 1..77: mol_type = other DNA
tggccgtggccgtgctcgtcctcgtcggccggcttgtcgacgacggcggtctccgtcgtcaggatcatccgggccac

SEQ ID NO: 19 - DNA, 77 bp, synthetic construct
  misc_feature 1..77: note = nucleotide sequence of Bxb1 attP
  source 1..77: mol_type = other DNA
tatggccgtgatgacctgtgtcttcgtggtttgtctggtcaaccaccgcggtctcagtggtgtacggtacaaaccca

SEQ ID NO: 20 - DNA, 273 bp, synthetic construct
  misc_feature 1..273: note = nucleotide sequence of phi C31 attB
  source 1..273: mol_type = other DNA
gatgtaggtcacggtctcgaagccgcggtgcgggtgccagggcgtgcccttgggctccccgggcgcgtactccacctcacccatctggtccatcatgatgaacgggtcgaggtggcggtagttgatcccggcgaacgcgcggcgcaccgggaagccctcgccctcgaaaccgctgggcgcggtggtcacggtgagcacgggacgtgcgacggcgtcggcgggtgcggatacgcggggcagcgtcagcgggttctcgacggtcacggcgggcat

SEQ ID NO: 21 - DNA, 57 bp, synthetic construct
  misc_feature 1..57: note = nucleotide sequence of R4 attB
  source 1..57: mol_type = other DNA
gcgcccaagttgcccatgaccatgccgaagcagtggtagaagggcaccggcagacac

SEQ ID NO: 22 - DNA, 32 bp, synthetic construct
  misc_feature 1..32: note = primer
  source 1..32: mol_type = other DNA
catgaatctagaagtgcaggtgccagaacatt

SEQ ID NO: 23 - DNA, 32 bp, synthetic construct
  misc_feature 1..32: note = primer
  source 1..32: mol_type = other DNA
catgaatcatgaccccctgaacctgaaacata

SEQ ID NO: 24 - DNA, 23 bp, synthetic construct
  misc_feature 1..23: note = target nucleotide sequence of gRNA-A1
  misc_feature 21..23: note = PAM sequence
  source 1..23: mol_type = other DNA
gggcccaggcgccgtttaatagg

SEQ ID NO: 25 - DNA, 23 bp, synthetic construct
  misc_feature 1..23: note = target nucleotide sequence of gRNA-B1
  misc_feature 21..23: note = PAM sequence
  source 1..23: mol_type = other DNA
tgccgcagagtgccaggtgcagg

SEQ ID NO: 26 - DNA, 23 bp, synthetic construct
  misc_feature 1..23: note = primer
  source 1..23: mol_type = other DNA
gagggcctatttcccatgattcc

SEQ ID NO: 27 - DNA, 25 bp, synthetic construct
  misc_feature 1..25: note = primer
  source 1..25: mol_type = other DNA
caccggggcccaggcgccgtttaat

SEQ ID NO: 28 - DNA, 25 bp, synthetic construct
  misc_feature 1..25: note = primer
  source 1..25: mol_type = other DNA
aaacattaaacggcgcctgggcccc

SEQ ID NO: 29 - DNA, 25 bp, synthetic construct
  misc_feature 1..25: note = primer
  source 1..25: mol_type = other DNA
caccgtgccgcagagtgccaggtgc

SEQ ID NO: 30 - DNA, 25 bp, synthetic construct
  misc_feature 1..25: note = primer
  source 1..25: mol_type = other DNA
aaacgcacctggcactctgcggcac

SEQ ID NO: 31 - DNA, 19 bp, synthetic construct
  misc_feature 1..19: note = primer
  source 1..19: mol_type = other DNA
gaactgaccgtctgctcca

SEQ ID NO: 32 - DNA, 20 bp, synthetic construct
  misc_feature 1..20: note = primer
  source 1..20: mol_type = other DNA
tgccgaagcagtggtagaag

SEQ ID NO: 33 - DNA, 20 bp, synthetic construct
  misc_feature 1..20: note = primer
  source 1..20: mol_type = other DNA
gggcaacgtgctggttattg

SEQ ID NO: 34 - DNA, 21 bp, synthetic construct
  misc_feature 1..21: note = primer
  source 1..21: mol_type = other DNA
gtgcccttctaccactgcttc

SEQ ID NO: 35 - DNA, 20 bp, synthetic construct
  misc_feature 1..20: note = primer
  source 1..20: mol_type = other DNA
agagtgaagcagaacgtggg

SEQ ID NO: 36 - DNA, 20 bp, synthetic construct
  misc_feature 1..20: note = primer
  source 1..20: mol_type = other DNA
tgctttttcgcaaccatggg

SEQ ID NO: 37 - DNA, 20 bp, synthetic construct
  misc_feature 1..20: note = primer
  source 1..20: mol_type = other DNA
ggggcgtacttggcatatga

SEQ ID NO: 38 - DNA, 20 bp, synthetic construct
  misc_feature 1..20: note = primer
  source 1..20: mol_type = other DNA
atgcagatcgagaagcacct

SEQ ID NO: 39 - DNA, 20 bp, synthetic construct
  misc_feature 1..20: note = primer
  source 1..20: mol_type = other DNA
aacgcaccagaccagcagac

SEQ ID NO: 40 - DNA, 19 bp, synthetic construct
  misc_feature 1..19: note = primer
  source 1..19: mol_type = other DNA
gacgtggggcctagaggct

SEQ ID NO: 41 - DNA, 20 bp, synthetic construct
  misc_feature 1..20: note = primer
  source 1..20: mol_type = other DNA
caggcggggaagattcagaa

SEQ ID NO: 42 - DNA, 20 bp, synthetic construct
  misc_feature 1..20: note = primer
  source 1..20: mol_type = other DNA
tagagagcctgggcctagag

SEQ ID NO: 43 - DNA, 20 bp, synthetic construct
  misc_feature 1..20: note = primer
  source 1..20: mol_type = other DNA
ccctcaaggtgtgaacaggg

SEQ ID NO: 44 - DNA, 20 bp, synthetic construct
  misc_feature 1..20: note = primer
  source 1..20: mol_type = other DNA
ctggagggaggcatgttctg

SEQ ID NO: 45 - DNA, 28 bp, synthetic construct
  misc_feature 1..28: note = primer
  source 1..28: mol_type = other DNA
ccaagcttcaggagaaagtgatggagtc

SEQ ID NO: 46 - DNA, 23 bp, synthetic construct
  misc_feature 1..23: note = primer
  source 1..23: mol_type = other DNA
caggtgcagctgcagcagtctgg

SEQ ID NO: 47 - DNA, 23 bp, synthetic construct
  misc_feature 1..23: note = primer
  source 1..23: mol_type = other DNA
caggtgcagctgcaggagtcggg

SEQ ID NO: 48 - DNA, 23 bp, synthetic construct
  misc_feature 1..23: note = primer
  source 1..23: mol_type = other DNA
gaggtgcagctgcaggagtctgg

SEQ ID NO: 49 - DNA, 31 bp, synthetic construct
  misc_feature 1..31: note = primer
  source 1..31: mol_type = other DNA
attatctgcagaagtctgacccgcacacagg

SEQ ID NO: 50 - DNA, 31 bp, synthetic construct
  misc_feature 1..31: note = primer
  source 1..31: mol_type = other DNA
attatctgcagtgtggagctggccaatgcat

SEQ ID NO: 51 - DNA, 33 bp, synthetic construct
  misc_feature 1..33: note = primer
  source 1..33: mol_type = other DNA
attatctgcagatggttatggttatggttatgg

SEQ ID NO: 52 - DNA, 31 bp, synthetic construct
  misc_feature 1..31: note = primer
  source 1..31: mol_type = other DNA
gtcggaagcttataaccacaaccataaccat

SEQ ID NO: 53 - DNA, 14 bp, Bos Taurus
  source 1..14: mol_type = unassigned DNA
tgtggagctggcca

SEQ ID NO: 54 - DNA, 48 bp, Homo sapiens
  source 1..48: mol_type = unassigned DNA
atgcttttgatatctggggccaagggacaatggtcaccgtctcttcag

SEQ ID NO: 55 - DNA, 46 bp, Bos Taurus
  source 1..46: mol_type = unassigned DNA
atggttatggttatggttatggttgtggttatggttatggttatac

SEQ ID NO: 56 - DNA, 44 bp, Homo sapiens
  source 1..44: mol_type = unassigned DNA
cttccagcactggggccagggcaccctggtcaccgtctcctcag

SEQ ID NO: 57 - DNA, 275 bp, Homo sapiens
  source 1..275: mol_type = unassigned DNA
gggggaggcttggtacagcctggggggtccctgagactctcctgtgcagcctctggattcacctttagcagctatgccatgagctgggtccgccaggctccagggaaggggctggagtgggtctcagctattagtggtagtggtggtagcacatactacgcagactccgtgaagggccggttcaccatctccagagacaattccaagaacacgctgtatctgcaaatgaacagcctgagagccgaggacacggccgtatattactgtgcgaaaga

SEQ ID NO: 58 - DNA, 43 bp, Bos Taurus
  source 1..43: mol_type = unassigned DNA
tagttgttatagtggttatggttatggttatggttgtggttat

SEQ ID NO: 59 - DNA, 286 bp, Homo sapiens
  source 1..286: mol_type = unassigned DNA
aggagtctggtcctacgctggtgaaacccacacagaccctcacgctgacctgcaccttctctgggttctcactcagcactagtggagtgggtgtgggctggatccgtcagcccccaggaaaggccctggagtggcttgcattcatttattgggatgatgataagcgctacagcccatctctgaagagcaggctcaccatcaccaaggacacctccaaaaaccaggtggtccttacaatgaccaacatggaccctgtggacacagccacatattactgtgcacacag

SEQ ID NO: 60 - DNA, 40 bp, Bos Taurus
  source 1..40: mol_type = unassigned DNA
ttgttatagtggttatggttatggttatggttgtggttat

SEQ ID NO: 61 - protein, 29 aa, synthetic construct
  REGION 1..29: note = Amino acid sequence of peptide comprising long CDRH3
GYGYGYGCGYGYGYTFQHWGQGTLVTVSS

SEQ ID NO: 62 - DNA, 20 bp, synthetic construct
  misc_feature 1..20: note = primer
  source 1..20: mol_type = other DNA
cacccacagtgtcacagagt

SEQ ID NO: 63 - DNA, 20 bp, synthetic construct
  misc_feature 1..20: note = primer
  source 1..20: mol_type = other DNA
tcactgtgggtggcaaaact

SEQ ID NO: 64 - DNA, 25 bp, synthetic construct
  misc_feature 1..25: note = primer
  source 1..25: mol_type = other DNA
cggtgtgcggttgtatgcctgctgt

SEQ ID NO: 65 - DNA, 25 bp, synthetic construct
  misc_feature 1..25: note = primer
  source 1..25: mol_type = other DNA
ggccaggcaggatgatggactccca

SEQ ID NO: 66 - DNA, 25 bp, synthetic construct
  misc_feature 1..25: note = primer
  source 1..25: mol_type = other DNA
cggttactattacacccacagcgtc

SEQ ID NO: 67 - DNA, 25 bp, synthetic construct
  misc_feature 1..25: note = primer
  source 1..25: mol_type = other DNA
ttgtagtggtggtgtctgctacacc

SEQ ID NO: 68 - DNA, 25 bp, synthetic construct
  misc_feature 1..25: note = primer
  source 1..25: mol_type = other DNA
gtagttactgtattcacacagtgac

SEQ ID NO: 69 - DNA, 20 bp, synthetic construct
  misc_feature 1..20: note = primer
  source 1..20: mol_type = other DNA
ctgcaggccctgtcctcttc

SEQ ID NO: 70 - DNA, 25 bp, synthetic construct
  misc_feature 1..25: note = primer
  source 1..25: mol_type = other DNA
atagtaataccactgtgggagggcc

SEQ ID NO: 71 - DNA, 28 bp, synthetic construct
  misc_feature 1..28: note = primer
  source 1..28: mol_type = other DNA
ccaagcttcaggagaaagtgatggagtc

SEQ ID NO: 72 - DNA, 23 bp, synthetic construct
  misc_feature 1..23: note = primer
  source 1..23: mol_type = other DNA
caggtgcagctgcagcagtctgg

SEQ ID NO: 73 - DNA, 23 bp, synthetic construct
  misc_feature 1..23: note = primer
  source 1..23: mol_type = other DNA
caggtgcagctgcaggagtcggg

SEQ ID NO: 74 - DNA, 23 bp, synthetic construct
  misc_feature 1..23: note = primer
  source 1..23: mol_type = other DNA
gaggtgcagctgcaggagtctgg

SEQ ID NO: 75 - DNA, 44 bp, synthetic construct
  misc_feature 1..44: note = nucleotide sequence of modified long DH chain substituted forhuman DH number 1-1
  source 1..44: mol_type = other DNA
gggcacaactggatggggctggctgggcaaacctatcggagctt

SEQ ID NO: 76 - DNA, 44 bp, synthetic construct
  misc_feature 1..44: note = nucleotide sequence of modified long DH chain substituted forhuman DH number 2-2
  source 1..44: mol_type = other DNA
cggcaggaatggctgggatattgtagccaccacaagcacccagt

SEQ ID NO: 77 - DNA, 44 bp, synthetic construct
  misc_feature 1..44: note = nucleotide sequence of modified long DH chain substituted forhuman DH number 3-3
  source 1..44: mol_type = other DNA
gtgtatcacaatctttggagtggtgatccctcagagcggcccct

SEQ ID NO: 78 - DNA, 44 bp, synthetic construct
  misc_feature 1..44: note = nucleotide sequence of modified long DH chain substituted forhuman DH number 4-4
  source 1..44: mol_type = other DNA
gcctgcagcagcttggttcagtgtatttaagcccccactgaatt

SEQ ID NO: 79 - DNA, 44 bp, synthetic construct
  misc_feature 1..44: note = nucleotide sequence of modified long DH chain substituted forhuman DH number 5-5
  source 1..44: mol_type = other DNA
gggcgatgacagcagcggctacagcatcaccgccatcgagtatt

SEQ ID NO: 80 - DNA, 44 bp, synthetic construct
  misc_feature 1..44: note = nucleotide sequence of modified long DH chain substituted forhuman DH number 6-6
  source 1..44: mol_type = other DNA
aggcccatacagctgggacgacagcccccaggacaattactata

SEQ ID NO: 81 - DNA, 62 bp, synthetic construct
  misc_feature 1..62: note = nucleotide sequence of modified long DH chain substituted forhuman DH number 1-7
  source 1..62: mol_type = other DNA
actgcacggccggaggatctacggcattgttgcattcaatgagtggttcacctacttctaca

SEQ ID NO: 82 - DNA, 44 bp, synthetic construct
  misc_feature 1..44: note = nucleotide sequence of modified long DH chain substituted forhuman DH number 2-8
  source 1..44: mol_type = other DNA
cagacaccacgacgtgttcatgctggtaccaatcgccggctggt

SEQ ID NO: 83 - DNA, 86 bp, synthetic construct
  misc_feature 1..86: note = nucleotide sequence of modified long DH chain substituted forhuman DH number 3-9
  source 1..86: mol_type = other DNA
cagcaagcacagactgcgggactacgtgctgtacgacgactacgggctgatcaactatcaggagtggaacgactacctggagttcc

SEQ ID NO: 84 - DNA, 83 bp, synthetic construct
  misc_feature 1..83: note = nucleotide sequence of modified long DH chain substituted forhuman DH number 3-10
  source 1..83: mol_type = other DNA
aagcaagcaccgcctgagagattacttcctgtacaacgagtatggccccaactacgaggagtggggcgactatctggcaaccc

SEQ ID NO: 85 - DNA, 59 bp, synthetic construct
  misc_feature 1..59: note = nucleotide sequence of modified long DH chain substituted forhuman DH number 4-11
  source 1..59: mol_type = other DNA
caagtcttgttgtggcggcaggagatactgcaacggagctgactgcttcaactgggact

SEQ ID NO: 86 - DNA, 62 bp, synthetic construct
  misc_feature 1..62: note = nucleotide sequence of modified long DH chain substituted forhuman DH number 5-12
  source 1..62: mol_type = other DNA
ccagctgggctacgacttctggtccggctactacaccgacaccctgtactactatttcggca

SEQ ID NO: 87 - DNA, 50 bp, synthetic construct
  misc_feature 1..50: note = nucleotide sequence of modified long DH chain substituted forhuman DH number 6-13
  source 1..50: mol_type = other DNA
cggcaagtactacgacttctggagcggctatcctcctggcgaggagtact

SEQ ID NO: 88 - DNA, 68 bp, synthetic construct
  misc_feature 1..68: note = nucleotide sequence of modified long DH chain substituted forhuman DH number 1-14
  source 1..68: mol_type = other DNA
gttccaggagagcggccctcctagactggatagatggtccggcaggaactactactactacagcggca

SEQ ID NO: 89 - DNA, 68 bp, synthetic construct
  misc_feature 1..68: note = nucleotide sequence of modified long DH chain substituted forhuman DH number 2-15
  source 1..68: mol_type = other DNA
tggcgaggagcacgaggtaccacagctgcactcctggagcggcagaaatctgtaccactatacaggcg

SEQ ID NO: 90 - DNA, 74 bp, synthetic construct
  misc_feature 1..74: note = nucleotide sequence of modified long DH chain substituted forhuman DH number 3-16
  source 1..74: mol_type = other DNA
agcaggcggccctgactacaggaacggctacaactactacgacttttacgatggctactacaactaccactaca

SEQ ID NO: 91 - DNA, 74 bp, synthetic construct
  misc_feature 1..74: note = nucleotide sequence of modified long DH chain substituted forhuman DH number 4-17
  source 1..74: mol_type = other DNA
ggcaggcggccccatctggcacgacgacgtgaagtactacgactttaacgatggctattacaattaccactaca

SEQ ID NO: 92 - DNA, 65 bp, synthetic construct
  misc_feature 1..65: note = nucleotide sequence of modified long DH chain substituted forhuman DH number 5-18
  source 1..65: mol_type = other DNA
tataccccccccttcggtattacggtattttgactggttaccccccagggagggttactacggta

SEQ ID NO: 93 - DNA, 62 bp, synthetic construct
  misc_feature 1..62: note = nucleotide sequence of modified long DH chain substituted forhuman DH number 6-19
  source 1..62: mol_type = other DNA
caccgactacaccatcgacgatgccggcatccactatcagggctctggcacattctggtact

SEQ ID NO: 94 - DNA, 62 bp, synthetic construct
  misc_feature 1..62: note = nucleotide sequence of modified long DH chain substituted forhuman DH number 1-20
  source 1..62: mol_type = other DNA
caccgactacaccatcgacgatcagggaaggttctaccagggcagcggcaccttctggtatt

SEQ ID NO: 95 - DNA, 53 bp, synthetic construct
  misc_feature 1..53: note = nucleotide sequence of modified long DH chain substituted forhuman DH number 2-21
  source 1..53: mol_type = other DNA
gaaccactacggctctggcagctacttttataggacagcctactactacgcca

SEQ ID NO: 96 - DNA, 47 bp, synthetic construct
  misc_feature 1..47: note = nucleotide sequence of modified long DH chain substituted forhuman DH number 3-22
  source 1..47: mol_type = other DNA
tattaggcggggaggaggggctcgctattactatcatgaggcagggg

SEQ ID NO: 97 - DNA, 62 bp, synthetic construct
  misc_feature 1..62: note = nucleotide sequence of modified long DH chain substituted forhuman DH number 4-23
  source 1..62: mol_type = other DNA
caagcacggcaggcgcatctatggcgtggttgcctttaaggagtggttcacctacttttaca

SEQ ID NO: 98 - DNA, 62 bp, synthetic construct
  misc_feature 1..62: note = nucleotide sequence of modified long DH chain substituted forhuman DH number 4-23
  source 1..62: mol_type = other DNA
cctgcacggcaagcgcatctatggcattgtggccctgggcgagctgttcacctacttttaca

SEQ ID NO: 99 - DNA, 47 bp, synthetic construct
  misc_feature 1..47: note = nucleotide sequence of modified long DH chain substituted forhuman DH number 6-25
  source 1..47: mol_type = other DNA
catgagacctgttgaccacggcatcgactacagcgggctgttcgtgt

SEQ ID NO: 100 - DNA, 59 bp, synthetic construct
  misc_feature 1..59: note = nucleotide sequence of modified long DH chain substituted forhuman DH number 1-26
  source 1..59: mol_type = other DNA
agggcaaggtgatagcagcagctggtacccccagggtttttactactactactacggta

SEQ ID NO: 101 - DNA, 17 bp, Homo sapiens
  source 1..17: mol_type = unassigned DNA
ggtacaactggaacgac

SEQ ID NO: 102 - DNA, 31 bp, Homo sapiens
  source 1..31: mol_type = unassigned DNA
aggatattgtagtagtaccagctgctatgcc

SEQ ID NO: 103 - DNA, 31 bp, Homo sapiens
  source 1..31: mol_type = unassigned DNA
gtattacgatttttggagtggttattatacc

SEQ ID NO: 104 - DNA, 16 bp, Homo sapiens
  source 1..16: mol_type = unassigned DNA
tgactacagtaactac

SEQ ID NO: 105 - DNA, 20 bp, Homo sapiens
  source 1..20: mol_type = unassigned DNA
gtggatacagctatggttac

SEQ ID NO: 106 - DNA, 18 bp, Homo sapiens
  source 1..18: mol_type = unassigned DNA
gagtatagcagctcgtcc

SEQ ID NO: 107 - DNA, 17 bp, Homo sapiens
  source 1..17: mol_type = unassigned DNA
ggtataactggaactac

SEQ ID NO: 108 - DNA, 31 bp, Homo sapiens
  source 1..31: mol_type = unassigned DNA
aggatattgtactaatggtgtatgctatacc

SEQ ID NO: 109 - DNA, 31 bp, Homo sapiens
  source 1..31: mol_type = unassigned DNA
gtattacgatattttgactggttattataac

SEQ ID NO: 110 - DNA, 31 bp, Homo sapiens
  source 1..31: mol_type = unassigned DNA
gtattactatggttcggggagttattataac

SEQ ID NO: 111 - DNA, 16 bp, Homo sapiens
  source 1..16: mol_type = unassigned DNA
tgactacagtaactac

SEQ ID NO: 112 - DNA, 23 bp, Homo sapiens
  source 1..23: mol_type = unassigned DNA
gtggatatagtggctacgattac

SEQ ID NO: 113 - DNA, 21 bp, Homo sapiens
  source 1..21: mol_type = unassigned DNA
gggtatagcagcagctggtac

SEQ ID NO: 114 - DNA, 17 bp, Homo sapiens
  source 1..17: mol_type = unassigned DNA
ggtataaccggaaccac

SEQ ID NO: 115 - DNA, 31 bp, Homo sapiens
  source 1..31: mol_type = unassigned DNA
aggatattgtagtggtggtagctgctactcc

SEQ ID NO: 116 - DNA, 37 bp, Homo sapiens
  source 1..37: mol_type = unassigned DNA
gtattatgattacgtttgggggagttatgcttatacc

SEQ ID NO: 117 - DNA, 16 bp, Homo sapiens
  source 1..16: mol_type = unassigned DNA
tgactacggtgactac

SEQ ID NO: 118 - DNA, 20 bp, Homo sapiens
  source 1..20: mol_type = unassigned DNA
gtggatacagctatggttac

SEQ ID NO: 119 - DNA, 21 bp, Homo sapiens
  source 1..21: mol_type = unassigned DNA
gggtatagcagtggctggtac

SEQ ID NO: 120 - DNA, 17 bp, Homo sapiens
  source 1..17: mol_type = unassigned DNA
ggtataactggaacgac

SEQ ID NO: 121 - DNA, 28 bp, Homo sapiens
  source 1..28: mol_type = unassigned DNA
agcatattgtggtggtgattgctattcc

SEQ ID NO: 122 - DNA, 31 bp, Homo sapiens
  source 1..31: mol_type = unassigned DNA
gtattactatgatagtagtggttattactac

SEQ ID NO: 123 - DNA, 19 bp, Homo sapiens
  source 1..19: mol_type = unassigned DNA
tgactacggtggtaactcc

SEQ ID NO: 124 - DNA, 20 bp, Homo sapiens
  source 1..20: mol_type = unassigned DNA
gtagagatggctacaattac

SEQ ID NO: 125 - DNA, 18 bp, Homo sapiens
  source 1..18: mol_type = unassigned DNA
gggtatagcagcggctac

SEQ ID NO: 126 - DNA, 20 bp, Homo sapiens
  source 1..20: mol_type = unassigned DNA
ggtatagtgggagctactac

SEQ ID NO: 127 - DNA, 31 bp, Bos taurus
  source 1..31: mol_type = unassigned DNA
agaataccgtgatgatggttactgctacacc

SEQ ID NO: 128 - DNA, 31 bp, Bos taurus
  source 1..31: mol_type = unassigned DNA
agaatatcgtgatgatggttactgctacacc

SEQ ID NO: 129 - DNA, 119 bp, Bos taurus
  source 1..119: mol_type = unassigned DNA
agactatcgtgatgatggttactgctacacccacagtgactcaggccctgacataaagtctgacccgcacacaggtgtggagctggccaatgcatccccaggggcactgggctcccaag

SEQ ID NO: 130 - DNA, 31 bp, Bos taurus; identical to SEQ ID NO: 128
  source 1..31: mol_type = unassigned DNA

SEQ ID NO: 131 - DNA, 16 bp, Bos taurus
  source 1..16: mol_type = unassigned DNA
ttactatagtgaccac

SEQ ID NO: 132 - DNA, 16 bp, Bos taurus
  source 1..16: mol_type = unassigned DNA
ttactatagtgaccac

SEQ ID NO: 133 - DNA, 16 bp, Bos taurus
  source 1..16: mol_type = unassigned DNA
ttactatagtgaccac

SEQ ID NO: 134 - DNA, 16 bp, Bos taurus
  source 1..16: mol_type = unassigned DNA
ttactatagtgaccac

SEQ ID NO: 135 - DNA, 36 bp, Bos taurus
  source 1..36: mol_type = unassigned DNA
gtattgtggtagctattgtggtagttattatggtac

SEQ ID NO: 136 - DNA, 36 bp, Bos taurus; identical to SEQ ID NO: 135
  source 1..36: mol_type = unassigned DNA

SEQ ID NO: 137 - DNA, 36 bp, Bos taurus; identical to SEQ ID NO: 135
  source 1..36: mol_type = unassigned DNA

SEQ ID NO: 138 - DNA, 43 bp, Bos taurus
  source 1..43: mol_type = unassigned DNA
gtagttatagtggttatggttatggttatagttatggttatac

SEQ ID NO: 139 - DNA, 42 bp, Bos taurus
  source 1..42: mol_type = unassigned DNA
atgatacgataggtgtggttgtagttattgtagtgttgctac

SEQ ID NO: 140 - DNA, 42 bp, Bos taurus
  source 1..42: mol_type = unassigned DNA
atgatacgataggtgtggttttagttattgtagtgttgctac

SEQ ID NO: 141 - DNA, 42 bp, Bos taurus; identical to SEQ ID NO: 140
  source 1..42: mol_type = unassigned DNA

SEQ ID NO: 142 - DNA, 58 bp, Bos taurus
  source 1..58: mol_type = unassigned DNA
gtagttgttatagtggttatggttatggttgtggttatggttatggttatgattatac

SEQ ID NO: 143 - DNA, 58 bp, Bos taurus
  source 1..58: mol_type = unassigned DNA
gtagttgttatagtggttatggttatggttatggttgtggttatggttatggttatac

SEQ ID NO: 144 - DNA, 58 bp, Bos taurus; identical to SEQ ID NO: 143
  source 1..58: mol_type = unassigned DNA

SEQ ID NO: 145 - DNA, 67 bp, Bos taurus
  source 1..67: mol_type = unassigned DNA
gtagttatggtggttatggttatggtggttatggttgttatggttatggttatggttatggttatac

SEQ ID NO: 146 - DNA, 73 bp, Bos taurus
  source 1..73: mol_type = unassigned DNA
gtagttatggtggttatggttatggtggttatggttgttatggttatggttatggttatggttatggttatac

SEQ ID NO: 147 - DNA, 148 bp, Bos taurus
  source 1..148: mol_type = unassigned DNA
gtagttgtcctgatggttatagttatggttatggttgtggttatggttatggttgtagtggttatgattgttatggttatggtggttatggtggttatggtggttatggttatagtagttatagttatagttatacttacgaatatac

SEQ ID NO: 148 - DNA, 14 bp, Bos taurus
  source 1..14: mol_type = unassigned DNA
gaactcggtggggc

SEQ ID NO: 149 - DNA, 14 bp, Bos taurus
  source 1..14: mol_type = unassigned DNA
gaactcggtggggc

SEQ ID NO: 150 - DNA, 17 bp, Macaca fascicularis
  source 1..17: mol_type = unassigned DNA
ggtataactggaactac

SEQ ID NO: 151 - DNA, 31 bp, Macaca fascicularis
  source 1..31: mol_type = unassigned DNA
agaatattgtagtagtacttactgctcctcc

SEQ ID NO: 152 - DNA, 42 bp, Macaca fascicularis
  source 1..42: mol_type = unassigned DNA
gtattacgaggatgattacggttactattacacccacagcgt

SEQ ID NO: 153 - DNA, 19 bp, Macaca fascicularis
  source 1..19: mol_type = unassigned DNA
tgactacggtagcagctac

SEQ ID NO: 154 - DNA, 20 bp, Macaca fascicularis
  source 1..20: mol_type = unassigned DNA
gtggatacagctacagttac

SEQ ID NO: 155 - DNA, 21 bp, Macaca fascicularis
  source 1..21: mol_type = unassigned DNA
gggtatagcagcggctggtac

SEQ ID NO: 156 - DNA, 17 bp, Macaca fascicularis
  source 1..17: mol_type = unassigned DNA
ggtatagctggaacgac

SEQ ID NO: 157 - DNA, 31 bp, Macaca fascicularis
  source 1..31: mol_type = unassigned DNA
agaatactgtactggtagtggttgctatgcc

SEQ ID NO: 158 - DNA, 22 bp, Macaca fascicularis
  source 1..22: mol_type = unassigned DNA
gtactggggtgattattatgac

SEQ ID NO: 159 - DNA, 31 bp, Macaca fascicularis
  source 1..31: mol_type = unassigned DNA
agcatattgtagtggtggtgtctgctacacc

SEQ ID NO: 160 - DNA, 35 bp, Macaca fascicularis
  source 1..35: mol_type = unassigned DNA
gtggatacagctacagttaccacagttttgccacc

SEQ ID NO: 161 - DNA, 20 bp, Macaca fascicularis
  source 1..20: mol_type = unassigned DNA
gtggatatagctacggttac

SEQ ID NO: 162 - DNA, 18 bp, Macaca fascicularis
  source 1..18: mol_type = unassigned DNA
gggtatagcagctggtcc

SEQ ID NO: 163 - DNA, 17 bp, Macaca fascicularis
  source 1..17: mol_type = unassigned DNA
ggtataactggaatgac

SEQ ID NO: 164 - DNA, 31 bp, Macaca fascicularis
  source 1..31: mol_type = unassigned DNA
agaatattgtagtggtatttactgctatgcc

SEQ ID NO: 165 - DNA, 16 bp, Macaca fascicularis
  source 1..16: mol_type = unassigned DNA
tgaatacagtaactac

SEQ ID NO: 166 - DNA, 16 bp, Macaca fascicularis
  source 1..16: mol_type = unassigned DNA
tgactacggtaactac

SEQ ID NO: 167 - DNA, 23 bp, Macaca fascicularis
  source 1..23: mol_type = unassigned DNA
ggggatacagtgggtacagttac

SEQ ID NO: 168 - DNA, 21 bp, Macaca fascicularis
  source 1..21: mol_type = unassigned DNA
gggtatagcggcagctggaac

SEQ ID NO: 169 - DNA, 17 bp, Macaca fascicularis
  source 1..17: mol_type = unassigned DNA
ggaacacctggaacgac

SEQ ID NO: 170 - DNA, 31 bp, Macaca fascicularis
  source 1..31: mol_type = unassigned DNA
agcacactgtagtgatagtggctgctcctcc

SEQ ID NO: 171 - DNA, 21 bp, Macaca fascicularis
  source 1..21: mol_type = unassigned DNA
gggtatagcggtggctggtcc

SEQ ID NO: 172 - DNA, 36 bp, Macaca fascicularis
  source 1..36: mol_type = unassigned DNA
gtattactatagtggtagttattactaccacagtgt

SEQ ID NO: 173 - DNA, 17 bp, Macaca fascicularis
  source 1..17: mol_type = unassigned DNA
gggtatagcagcagcta

SEQ ID NO: 174 - DNA, 21 bp, Macaca fascicularis
  source 1..21: mol_type = unassigned DNA
gggtatagcagcggctggtcc

SEQ ID NO: 175 - DNA, 20 bp, Macaca fascicularis
  source 1..20: mol_type = unassigned DNA
ggtatagtgggaactacaac